European Patent Application EP 4 234 580 A1, published August 30, 2023. Title: NKG2A-targeting antibody and use thereof. Applicant: Bioheng Therapeutics Limited. The sequence listing filed with the application follows.

SEQUENCE LISTING (38 sequences)

SEQ ID NO: 1 - protein, 11 aa, Artificial Sequence
  CDR-L1
SASSSVSSYIY

SEQ ID NO: 2 - protein, 7 aa, Artificial Sequence
  CDR-L2
LTSNLAS

SEQ ID NO: 3 - protein, 9 aa, Artificial Sequence
  CDR-L3
QQWSGNPYT

SEQ ID NO: 4 - protein, 7 aa, Artificial Sequence
  CDR-H1
GFTFSSY

SEQ ID NO: 5 - protein, 6 aa, Artificial Sequence
  CDR-H2
SSGGSY

SEQ ID NO: 6 - protein, 10 aa, Artificial Sequence
  CDR-H3
HGDYPRFFDV

SEQ ID NO: 7 - protein, 107 aa, Artificial Sequence
  hZ199 VL
EIVLTQSPATLSLSPGERATLSCSASSSVSSYIYWYQQKPGQAPRLLIYLTSNLASGIPARFSGSGSGTDFTLTISSLEPEDFAVYYCQQWSGNPYTFGQGTKLEIK

SEQ ID NO: 8 - protein, 119 aa, Artificial Sequence
  hZ199 VH
EVQLVESGGGLVKPGGSLRLSCAASGFTFSSYAKSWVRQAPGKGLEWVSEISSGGSYTYYADSVKGRFTISRDNAKNSLYLQMNSLRAEDTAVYYCARHGDYPRFFDVWGQGTTVTVSS

SEQ ID NO: 9 - protein, 244 aa, Artificial Sequence
  hZ199 scFv
EIVLTQSPATLSLSPGERATLSCSASSSVSSYIYWYQQKPGQAPRLLIYLTSNLASGIPARFSGSGSGTDFTLTISSLEPEDFAVYYCQQWSGNPYTFGQGTKLEIKGSTSGSGKPGSGEGSTKGEVQLVESGGGLVKPGGSLRLSCAASGFTFSSYAKSWVRQAPGKGLEWVSEISSGGSYTYYADSVKGRFTISRDNAKNSLYLQMNSLRAEDTAVYYCARHGDYPRFFDVWGQGTTVTVSS

SEQ ID NO: 10 - protein, 107 aa, Artificial Sequence
  hZ199-V1 VL
EIVLTQSPATLSLSPGERATMSCSASSSVSSYIYWYQQKPGQAPRLLIYLTSNLASGVPARFSGSGSGTDFTLTISSLEPEDFATYYCQQWSGNPYTFGQGTKLEIK

SEQ ID NO: 11 - protein, 119 aa, Artificial Sequence
  hZ199-V1 VH
EVQLVESGGGLVKPGGSLRLSCAASGFTFSSYAMSWVRQAPGKGLEWVAEISSGGSYTYYPDSVKGRFTISRDNAKNSLYLQMNSLRAEDTAVYYCTRHGDYPRFFDVWGQGTTVTVSS

SEQ ID NO: 12 - protein, 244 aa, Artificial Sequence
  hZ199-V1 scFv
EIVLTQSPATLSLSPGERATMSCSASSSVSSYIYWYQQKPGQAPRLLIYLTSNLASGVPARFSGSGSGTDFTLTISSLEPEDFATYYCQQWSGNPYTFGQGTKLEIKGSTSGSGKPGSGEGSTKGEVQLVESGGGLVKPGGSLRLSCAASGFTFSSYAMSWVRQAPGKGLEWVAEISSGGSYTYYPDSVKGRFTISRDNAKNSLYLQMNSLRAEDTAVYYCTRHGDYPRFFDVWGQGTTVTVSS

SEQ ID NO: 13 - protein, 107 aa, Artificial Sequence
  hZ199-V2 VL
EIVLTQSPATLSLSPGERATMTCSASSSVSSYIYWYQQKPGQAPRLLIYLTSNLASGIPARFSGSGSGTDFTLTISSLEPEDFATYYCQQWSGNPYTFGQGTKVEIK

SEQ ID NO: 14 - protein, 244 aa, Artificial Sequence
  hZ199-V2 scFv
EIVLTQSPATLSLSPGERATMTCSASSSVSSYIYWYQQKPGQAPRLLIYLTSNLASGIPARFSGSGSGTDFTLTISSLEPEDFATYYCQQWSGNPYTFGQGTKVEIKGSTSGSGKPGSGEGSTKGEVQLVESGGGLVKPGGSLRLSCAASGFTFSSYAMSWVRQAPGKGLEWVAEISSGGSYTYYPDSVKGRFTISRDNAKNSLYLQMNSLRAEDTAVYYCTRHGDYPRFFDVWGQGTTVTVSS

SEQ ID NO: 15 - DNA, 732 bp, Artificial Sequence
  hZ199-V1
gaaatagtcctgactcagtctccggcaactttgtctttgtcacctggagaacgcgctacaatgtcctgctccgcgtcctctagcgtttcaagctacatatactggtaccaacaaaagccgggtcaagccccgcgcctgctgatctatctcaccagcaacctcgcgtccggtgtgcctgctcgattcagcggttctgggtctgggacggacttcactctcactatttcaagcctcgaaccagaggacttcgctacttactattgtcagcaatggagtgggaacccgtacacgttcggacaaggaactaagctcgagattaaaggtagtaccagcggatctgggaagcctggtagtggagagggcagcacaaagggtgaggtgcagttggtagaatcaggtgggggactcgtgaaacccggcggatcattgaggctcagttgcgccgcatctggattcacgtttagttcctacgccatgtcatgggtcaggcaagcccctggaaaaggccttgagtgggttgctgaaatttccagcgggggtagctacacttactacccggatagcgttaaaggcagattcactattagtagggataacgccaagaacagtctttacctccagatgaattcccttagggctgaagatacagcggtctactactgtacaaggcacggggactatccccgcttcttcgatgtatggggacaaggcacgcttgtgacagtgagcagc

SEQ ID NO: 16 - DNA, 732 bp, Artificial Sequence
  hZ199-V2
gaaatagtcttgacccagtctcccgctaccctcagtctttcacccggtgaacgcgctacgatgacgtgttcagcatccagctctgtgtcttcctacatttattggtaccagcagaaaccaggccaagcgccgcgcctcctcatttaccttacttcaaaccttgcatccggtattcccgcgagattcagcggtagtggttctggaacggattttacacttacgattagttcacttgaacccgaagatttcgccacgtattactgtcagcaatggtcaggaaatccttacactttcggccaaggtaccaaagtcgagatcaaagggtccacttctggttcaggtaagccaggtagtggcgaggggagtacaaagggggaagtgcagctcgtcgagtcaggtggcggacttgtaaaaccgggggggtcactccggctgtcctgcgcagcgagtggatttacctttagcagttatgcaatgtcctgggtaagacaagctccgggcaagggactggaatgggtggctgaaatctctagtggtggaagttatacctactaccctgatagcgtgaagggtagatttactattagtcgggacaacgctaagaatagcttgtaccttcaaatgaacagtttgcgagcagaggacactgcagtttattattgcacccggcacggagattatcctcgcttttttgacgtatggggacagggaactctcgtgactgttagtagc

SEQ ID NO: 17 - protein, 25 aa, Artificial Sequence
  CD8alpha transmembrane domain
IYIWAPLAGTCGVLLLSLVITLYCK

SEQ ID NO: 18 - DNA, 75 bp, Artificial Sequence
  CD8alpha transmembrane domain
atctacatctgggcgcccttggccgggacttgtggggtccttctcctgtcactggttatcaccctttactgcaaa

SEQ ID NO: 19 - protein, 27 aa, Artificial Sequence
  CD28 transmembrane domain
FWVLVVVGGVLACYSLLVTVAFIIFWV

SEQ ID NO: 20 - DNA, 81 bp, Artificial Sequence
  CD28 transmembrane domain
ttttgggtcctcgtcgtagttggaggggtacttgcctgttatagcctcctggttaccgtagcatttattatattctgggtg

SEQ ID NO: 21 - protein, 41 aa, Artificial Sequence
  CD28 costimulatory domain
RSKRSRLLHSDYMNMTPRRPGPTRKHYQPYAPPRDFAAYRS

SEQ ID NO: 22 - DNA, 123 bp, Artificial Sequence
  CD28 costimulatory domain
aggagtaagaggagcaggctcctgcacagtgactacatgaacatgactccccgccgccccgggcccacccgcaagcattaccagccctatgccccaccacgcgacttcgcagcctatcgctcc

SEQ ID NO: 23 - protein, 40 aa, Artificial Sequence
  4-1BB costimulatory domain
RGRKKLLYIFKQPFMRPVQTTQEEDGCSCRFPEEEEGGCE

SEQ ID NO: 24 - DNA, 120 bp, Artificial Sequence
  4-1BB costimulatory domain
cggggcagaaagaaactcctgtatatattcaaacaaccatttatgagaccagtacaaactactcaagaggaagatggctgtagctgccgatttccagaagaagaagaaggaggatgtgaa

SEQ ID NO: 25 - protein, 113 aa, Artificial Sequence
  4-1BB costimulatory domain
LRVKFSRSADAPAYQQGQNQLYNELNLGRREEYDVLDKRRGRDPEMGGKPRRKNPQEGLYNELQKDKMAEAYSEIGMKGERRRGKGHDGLYQGLSTATKDTYDALHMQALPPR

SEQ ID NO: 26 - DNA, 339 bp, Artificial Sequence
  CD3zeta signaling domain
ctgagagtgaagttcagcaggagcgcagacgcccccgcgtaccagcagggccagaaccagctctataacgagctcaatctaggacgaagagaggagtacgatgttttggacaagagacgtggccgggaccctgagatggggggaaagccgagaaggaagaaccctcaggaaggcctgtacaatgaactgcagaaagataagatggcggaggcctacagtgagattgggatgaaaggcgagcgccggaggggcaaggggcacgatggcctttaccagggtctcagtacagccaccaaggacacctacgacgcccttcacatgcaggccctgccccctcgc

SEQ ID NO: 27 - protein, 114 aa, Artificial Sequence
  CD3zeta signaling domain
LRVKFSRSADAPAYQQGQNQLFNELNLGRREEFDVLDKRRGRDPEMGGKPQRRKNPQEGLYNELQKDKMAEAYSEIGMKGERRRGKGHDGLFQGLSTATKDTFDALHMQALPPR

SEQ ID NO: 28 - DNA, 342 bp, Artificial Sequence
  CD3zeta signaling domain
ctgagagtgaagttcagcaggagcgcagacgcccccgcgtaccagcagggccagaaccagctctttaacgagctcaatctaggacgaagagaggagttcgatgttttggacaagagacgtggccgggaccctgagatggggggaaagccgcagagaaggaagaaccctcaggaaggcctgtacaatgaactgcagaaagataagatggcggaggcctacagtgagattgggatgaaaggcgagcgccggaggggcaaggggcacgatggccttttccagggtctcagtacagccaccaaggacacctttgacgcccttcacatgcaggccctgccccctcgc

SEQ ID NO: 29 - protein, 20 aa, Artificial Sequence
  B2M signal peptide
MSRSVALAVLALLSLSGLEA

SEQ ID NO: 30 - DNA, 60 bp, Artificial Sequence
  B2M signal peptide
atgtcccgctctgttgctttggctgtgctggcccttttgtcccttagcggactggaggcc

SEQ ID NO: 31 - protein, 21 aa, Artificial Sequence
  CD8alpha signal peptide
MALPVTALLLPLALLLHAARP

SEQ ID NO: 32 - DNA, 63 bp, Artificial Sequence
  CD8alpha signal peptide
atggccttaccagtgaccgccttgctcctgccgctggccttgctgctccacgccgccaggccg

SEQ ID NO: 33 - protein, 45 aa, Artificial Sequence
  CD8alpha hinge region
TTTPAPRPPTPAPTIASQPLSLRPEACRPAAGGAVHTRGLDFACD

SEQ ID NO: 34 - DNA, 135 bp, Artificial Sequence
  CD8alpha hinge region
accacgacgccagcgccgcgaccaccaacaccggcgcccaccatcgcgtcgcagcccctgtccctgcgcccagaggcgtgccggccagcggcggggggcgcagtgcacacgagggggctggacttcgcctgtgat

SEQ ID NO: 35 - protein, 39 aa, Artificial Sequence
  CD28 hinge region
IEVMYPPPYLDNEKSNGTIIHVKGKHLCPSPLFPGPSKP

SEQ ID NO: 36 - DNA, 117 bp, Artificial Sequence
  CD28 hinge region
attgaagttatgtatcctcctccttacctagacaatgagaagagcaatggaaccattatccatgtgaaagggaaacacctttgtccaagtcccctatttcccggaccttctaagccc

SEQ ID NO: 37 - protein, 12 aa, Artificial Sequence
  IgG4 hinge region
ESKYGPPCPPCP

SEQ ID NO: 38 - DNA, 36 bp, Artificial Sequence
  IgG4 hinge region
gaaagcaaatacgggccgccgtgtccaccctgtccg